European Patent Specification EP 3 739 044 B1, published July 12, 2023. Title: VARIANT PHOSPHORIBOSYLPYROPHOSPHATE AMIDOTRANSFERASE AND METHOD OF PREPARING PURINE NUCLEOTIDE USING THE SAME. Applicant: CJ CheilJedang Corporation. The sequence listing filed with the application follows.

SEQUENCE LISTING (24 sequences)

SEQ ID NO: 1 - DNA, 1500 bp, Unknown
  purF
gtggtgaacactactttccccagcgacgtgaatttagatgaccaaggcgagcaagaaccccgcgaagagtgcggtgtctttggcgtctgggctcctggtgaagatgttgcgacactgacctactttggtctgttcgcattgcagcatcgtgggcaggaagctgcaggtatcggcgtcggtgatggagaccgcctcgttgtcttcaaagacatgggcttggtctcgaatattttcgatgagtccattttaaattccctccatggctccgtgggcgtggggcatacgcgctactcgactgccggtggcaaagagtggtcgaatgtccagccgatgtttaataccacctcaaatggggtagacatcgctttgtgccacaacggcaacttggtgaactaccaagaactgcgcgatgaagcagtagctctgggactttaccgagagaatgaaaaatccctgtcggattccatgatcatgacagctttgctggcgcacggagtcggggaaggcaactctgtctttgacgccgctaagcaactgctgccaagcatcaaaggcgctttttgcttgacctttaccgatggcaagaccttgtacgccgcgcgtgacccgcacggtgtacgccccttggtcattggccgcttggcgcaaggctgggttgttgcttccgaaacctgtgcgctggatatcgtgggcgcacagtttatccgtgaggtagagcccggtgaacttatctctgtcaatgaggcaggaatccacagcgaaaaattcgctgagccgaagcgccagggctgcgtctttgaatacgtctacttggcacgtccagacaccgtgatcaaaggccgcaacgttcacgcgacgcgcgtggatattggtcgcgcacttgcgaaatctcaccctgcgccagaagctgacatggtcatccccgtgccagaatccggaaacccggcagctgttggctacgcccgggaatcgggcctgacatttgcgcacggcttggtcaaaaacgcctacgtgggtcgaaccttcattcagcccacccagaccttgcgccagctgggtattcgcctcaagctcaaccccctgcgcgaggtcatcgagggcaagtcactcgttgttgtagatgactctattgtccgcggcaacacccaacgcgcgctggtgcgcatgctgcgtgaagcaggcgctgctgaagtgcacgtgcgcattgcttcaccgccagtcaaatggccttgtttctacggcattgacttcgcctcgcctggtgaattgattgctaatatcaagccttctgatgatcctcaggtagtaaccgatgcagtgtgcgaagctatcggagcagactctttagggtttgtatctgtagatgagatggttgaggcaacgcaccaacctatcaattccttgtgtaccgcttgctttgatggcaactacgaactcggacttccgaccgctaaccccaatgctgacgctgtgcgaactttgctcagccaaaagaactga

SEQ ID NO: 2 - protein, 499 aa, Unknown
  purF
MVNTTFPSDVNLDDQGEQEPREECGVFGVWAPGEDVATLTYFGLFALQHRGQEAAGIGVGDGDRLVVFKDMGLVSNIFDESILNSLHGSVGVGHTRYSTAGGKEWSNVQPMFNTTSNGVDIALCHNGNLVNYQELRDEAVALGLYRENEKSLSDSMIMTALLAHGVGEGNSVFDAAKQLLPSIKGAFCLTFTDGKTLYAARDPHGVRPLVIGRLAQGWVVASETCALDIVGAQFIREVEPGELISVNEAGIHSEKFAEPKRQGCVFEYVYLARPDTVIKGRNVHATRVDIGRALAKSHPAPEADMVIPVPESGNPAAVGYARESGLTFAHGLVKNAYVGRTFIQPTQTLRQLGIRLKLNPLREVIEGKSLVVVDDSIVRGNTQRALVRMLREAGAAEVHVRIASPPVKWPCFYGIDFASPGELIANIKPSDDPQVVTDAVCEAIGADSLGFVSVDEMVEATHQPINSLCTACFDGNYELGLPTANPNADAVRTLLSQKN

SEQ ID NO: 3 - DNA, 29 bp, Artificial Sequence
  purA a1t-1
gctctagaggccacgatgcccggagcatc

SEQ ID NO: 4 - DNA, 37 bp, Artificial Sequence
  purA a1t-2
taacgatagctgccaaggttattcacttcctagattt

SEQ ID NO: 5 - DNA, 37 bp, Artificial Sequence
  purA a1t-3
aggaagtgaataaccttggcagctatcgttatcgtcg

SEQ ID NO: 6 - DNA, 29 bp, Artificial Sequence
  purA a1t-4
gctctagaggtcacgaatgggtaggtgcc

SEQ ID NO: 7 - DNA, 29 bp, Artificial Sequence
  guaB a1t-1
gctctagactacgacaacacggtgcctaa

SEQ ID NO: 8 - DNA, 37 bp, Artificial Sequence
  guaB a1t-2
cacgattttcggtcaatacgggtcttctccttcgcac

SEQ ID NO: 9 - DNA, 36 bp, Artificial Sequence
  guaB a1t-3
aggagaagacccgtattgaccgaaaatcgtgtttct

SEQ ID NO: 10 - DNA, 29 bp, Artificial Sequence
  guaB a1t-4
gctctagaatcgacaagcaagcctgcacg

SEQ ID NO: 11 - DNA, 20 bp, Artificial Sequence
  purF tempF
aagttgatgcttcaggcaca

SEQ ID NO: 12 - DNA, 20 bp, Artificial Sequence
  purF tempR
tgcaaggattggctctttgt

SEQ ID NO: 13 - DNA, 19 bp, Artificial Sequence
  purF lib F
acacgagatagcccagtgg

SEQ ID NO: 14 - DNA, 20 bp, Artificial Sequence
  purF lib R
tcgtagttgccatcaaagca

SEQ ID NO: 15 - DNA, 19 bp, Artificial Sequence
  purF seq F
acacgagatagcccagtgg

SEQ ID NO: 16 - DNA, 21 bp, Artificial Sequence
  purF seq R
accaagtcatcgacgcacatt

SEQ ID NO: 17 - DNA, 30 bp, Artificial Sequence
  purF V2M 1F
gggtctagaagtactgacccgaccactgca

SEQ ID NO: 18 - DNA, 27 bp, Artificial Sequence
  purF V2M 1R
tggggaaagtagtgttcatcacgacgc

SEQ ID NO: 19 - DNA, 27 bp, Artificial Sequence
  purF V2M 2F
tagtagaatcagcgtcgtgatgaacac

SEQ ID NO: 20 - DNA, 30 bp, Artificial Sequence
  purF V2M 2R
gggtctagatggattcctgcctcattgaca

SEQ ID NO: 21 - DNA, 30 bp, Artificial Sequence
  purF G445R 1F
gggtctagaccgatggcaagaccttgtacg

SEQ ID NO: 22 - DNA, 31 bp, Artificial Sequence
  purF G445R 1R
caaaccctaaagagtctgctctgatagcttc

SEQ ID NO: 23 - DNA, 30 bp, Artificial Sequence
  purF G445R 2F
cagtgtgcgaagctatcagagcagactctt

SEQ ID NO: 24 - DNA, 32 bp, Artificial Sequence
  purF G445R 2R
gggtctagacaaggtcatcgatgtagccatcg